European Patent Application EP 4 335 851 A2, published March 13, 2024. Title: Pharmaceutical formulations and methods of use thereof. Applicant: ImmunoGen, Inc. The sequence listing filed with the application follows.

SEQUENCE LISTING (15 sequences)

SEQ ID NO: 1 - protein, 5 aa, synthetic construct
SSIMH

SEQ ID NO: 2 - protein, 17 aa, synthetic construct
YIKPYNDGTKYNEKFKG

SEQ ID NO: 3 - protein, 12 aa, synthetic construct
EGGNDYYDTMDY

SEQ ID NO: 4 - protein, 11 aa, synthetic construct
RASQDINSYLS

SEQ ID NO: 5 - protein, 7 aa, synthetic construct
RVNRLVD

SEQ ID NO: 6 - protein, 9 aa, synthetic construct
LQYDAFPYT

SEQ ID NO: 7 - protein, 121 aa, synthetic construct
  VARIANT 2: note = X is selected from phenylalanine or valine
QXQLVQSGAEVKKPGASVKVSCKASGYIFTSSIMHWVRQAPGQGLEWIGYIKPYNDGTKYNEKFKGRATLTSDRSTSTAYMELSSLRSEDTAVYYCAREGGNDYYDTMDYWGQGTLVTVSS

SEQ ID NO: 8 - protein, 121 aa, synthetic construct
QVQLVQSGAEVKKPGASVKVSCKASGYGFTSSIMHWVRQAPGQGLEWMGYIKPYNDGTKYNEKFKGRVTMTRDTSTSTVYMELSSLRSEDTAVYYCAREGGNDYYDTMDYWGQGTLVTVSS

SEQ ID NO: 9 - protein, 108 aa, synthetic construct
DIQMTQSPSSLSASVGDRVTITCRASQDINSYLSWFQQKPGKAPKTLIYRVNRLVDGVPSRFSGSGSGNDYTLTISSLQPEDFATYYCLQYDAFPYTFGQGTKVEIKR

SEQ ID NO: 10 - protein, 108 aa, synthetic construct
DIQMTQSPSSLSASVGDRVTITCRASQDINSYLAWFQQKPGKAPKSLIYRVNRLVSGVPSRFSGSGSGTDFTLTISSLQPEDFATYYCLQYDAFPYTFGQGTKVEIKR

SEQ ID NO: 11 - protein, 450 aa, synthetic construct
  VARIANT 2: note = X is selected from phenylalanine or valine
QXQLVQSGAEVKKPGASVKVSCKASGYIFTSSIMHWVRQAPGQGLEWIGYIKPYNDGTKYNEKFKGRATLTSDRSTSTAYMELSSLRSEDTAVYYCAREGGNDYYDTMDYWGQGTLVTVSSASTKGPSVFPLAPSSKSTSGGTAALGCLVKDYFPEPVTVSWNSGALTSGVHTFPAVLQSSGLYSLSSVVTVPSSSLGTQTYICNVNHKPSNTKVDKKVEPKSCDKTHTCPPCPAPELLGGPSVFLFPPKPKDTLMISRTPEVTCVVVDVSHEDPEVKFNWYVDGVEVHNAKTKPREEQYNSTYRVVSVLTVLHQDWLNGKEYKCKVSNKALPAPIEKTISKAKGQPREPQVYTLPPSRDELTKNQVSLTCLVKGFYPSDIAVEWESNGQPENNYKTTPPVLDSDGSFFLYSKLTVDKSRWQQGNVFSCSVMHEALHNHYTQKSLSLSPG

SEQ ID NO: 12 - protein, 450 aa, synthetic construct
  VARIANT 2: note = X is selected from phenylalanine or valine
QXQLVQSGAEVKKPGASVKVSCKASGYIFTSSIMHWVRQAPGQGLEWIGYIKPYNDGTKYNEKFKGRATLTSDRSTSTAYMELSSLRSEDTAVYYCAREGGNDYYDTMDYWGQGTLVTVSSASTKGPSVFPLAPSSKSTSGGTAALGCLVKDYFPEPVTVSWNSGALTSGVHTFPAVLQSSGLYSLSSVVTVPSSSLGTQTYICNVNHKPSNTKVDKKVEPKSCDKTHTCPPCPAPELLGGPSVFLFPPKPKDTLMISRTPEVTCVVVDVSHEDPEVKFNWYVDGVEVHNAKTKPREEQYNSTYRVVSVLTVLHQDWLNGKEYKCKVSNKALPAPIEKTISKAKGQPREPQVYTLPPSRDELTKNQVSLTCLVKGFYPSDIAVEWESNGQPENNYKTTPPVLDSDGSFFLYSKLTVDKSRWQQGNVFSCSVMHEALHNHYTQKSLCLSPG

SEQ ID NO: 13 - protein, 450 aa, synthetic construct
QVQLVQSGAEVKKPGASVKVSCKASGYGFTSSIMHWVRQAPGQGLEWMGYIKPYNDGTKYNEKFKGRVTMTRDTSTSTVYMELSSLRSEDTAVYYCAREGGNDYYDTMDYWGQGTLVTVSSASTKGPSVFPLAPSSKSTSGGTAALGCLVKDYFPEPVTVSWNSGALTSGVHTFPAVLQSSGLYSLSSVVTVPSSSLGTQTYICNVNHKPSNTKVDKKVEPKSCDKTHTCPPCPAPELLGGPSVFLFPPKPKDTLMISRTPEVTCVVVDVSHEDPEVKFNWYVDGVEVHNAKTKPREEQYNSTYRVVSVLTVLHQDWLNGKEYKCKVSNKALPAPIEKTISKAKGQPREPQVYTLPPSRDELTKNQVSLTCLVKGFYPSDIAVEWESNGQPENNYKTTPPVLDSDGSFFLYSKLTVDKSRWQQGNVFSCSVMHEALHNHYTQKSLSLSPG

SEQ ID NO: 14 - protein, 214 aa, synthetic construct
DIQMTQSPSSLSASVGDRVTITCRASQDINSYLSWFQQKPGKAPKTLIYRVNRLVDGVPSRFSGSGSGNDYTLTISSLQPEDFATYYCLQYDAFPYTFGQGTKVEIKRTVAAPSVFIFPPSDEQLKSGTASVVCLLNNFYPREAKVQWKVDNALQSGNSQESVTEQDSKDSTYSLSSTLTLSKADYEKHKVYACEVTHQGLSSPVTKSFNRGEC

SEQ ID NO: 15 - protein, 214 aa, synthetic construct
DIQMTQSPSSLSASVGDRVTITCRASQDINSYLAWFQQKPGKAPKSLIYRVNRLVSGVPSRFSGSGSGTDFTLTISSLQPEDFATYYCLQYDAFPYTFGQGTKVEIKRTVAAPSVFIFPPSDEQLKSGTASVVCLLNNFYPREAKVQWKVDNALQSGNSQESVTEQDSKDSTYSLSSTLTLSKADYEKHKVYACEVTHQGLSSPVTKSFNRGEC